European Patent Specification EP 3 712 240 B1, published September 27, 2023. Title: COMPOSITIONS FOR PRODUCING GLUCOSE SYRUPS. Applicant: Novozymes A/S. The sequence listing filed with the application follows.

SEQUENCE LISTING (25 sequences)

SEQ ID NO: 1 - protein, 616 aa, Aspergillus niger
ATLDSWLSNEATVARTAILNNIGADGAWVSGADSGIVVASPSTDNPDYFYTWTRDSGLVLKTLVDLFRNGDTSLLSTIENYISAQAIVQGISNPSGDLSSGAGLGEPKFNVDETAYTGSWGRPQRDGPALRATAMIGFGQWLLDNGYTSTATDIVWPLVRNDLSYVAQYWNQTGYDLWEEVNGSSFFTIAVQHRALVEGSAFATAVGSSCSWCDSQAPEILCYLQSFWTGSFILANFDSSRSGKDANTLLGSIHTFDPEAACDDSTFQPCSPRALANHKEVVDSFRSIYTLNDGLSDSEAVAVGRYPEDTYYNGNPWFLCTLAAAEQLYDALYQWDKQGSLEVTDVSLDFFKALYSDAATGTYSSSSSTYSSIVDAVKTFADGFVSIVETHAASNGSMSEQYDKSDGEQLSARDLTWSYAALLTANNRRNSVVPASWGETSASSVPGTCAATSAIGTYSSVTVTSWPSIVATGGTTTTATPTGSGSVTSTSKTTATASKTSTSTSSTSCTTPTAVAVTFDLTATTTYGENIYLVGSISQLGDWETSDGIALSADKYTSSDPLWYVTVTLPAGESFEYKFIRIESDDSVEWESDPNREYTVPQACGTSTATVTDTWR

SEQ ID NO: 2 - protein, 484 aa, Aspergillus niger
LSAAEWRTQSIYFLLTDRFGRTDNSTTATCDTGDQIYCGGSWQGIINHLDYIQGMGFTAIWISPITEQLPQDTADGEAYHGYWQQKIYDVNSNFGTADDLKSLSDALHARGMYLMVDVVPNHMGYAGNGNDVDYSVFDPFDSSSYFHPYCLITDWDNLTMVQDCWEGDTIVSLPDLNTTETAVRTIWYDWVADLVSNYSVDGLRIDSVLEVEPDFFPGYQEAAGVYCVGEVDNGNPALDCPYQKVLDGVLNYPIYWQLLYAFESSSGSISNLYNMIKSVASDCSDPTLLGNFIENHDNPRFASYTSDYSQAKNVLSYIFLSDGIPIVYAGEEQHYSGGKVPYNREATWLSGYDTSAELYTWIATTNAIRKLAISADSAYITYANDAFYTDSNTIAMRKGTSGSQVITVLSNKGSSGSSYTLTLSGSGYTSGTKLIEAYTCTSVTVDSSGDIPVPMASGLPRVLLPASVVDSSSLCGGSGRLYVE

SEQ ID NO: 3 - protein, 928 aa, Bacillus deramificans
DGNTTTIIVHYFRPAGDYQPWSLWMWPKDGGGAEYDFNQPADSFGAVASADIPGNPSQVGIIVRTQDWTKDVSADRYIDLSKGNEVWLVEGNSQIFYNEKDAEDAAKPAVSNAYLDASNQVLVKLSQPLTLGEGASGFTVHDDTANKDIPVTSVKDASLGQDVTAVLAGTFQHIFGGSDWAPDNHSTLLKKVTNNLYQFSGDLPEGNYQYKVALNDSWNNPSYPSDNINLTVPAGGAHVTFSYIPSTHAVYDTINNPNADLQVESGVKTDLVTVTLGEDPDVSHTLSIQTDGYQAKQVIPRNVLNSSQYYYSGDDLGNTYTQKATTFKVWAPTSTQVNVLLYDSATGSVTKIVPMTASGHGVWEATVNQNLENWYYMYEVTGQGSTRTAVDPYATAIAPNGTRGMIVDLAKTDPAGWNSDKHITPKNIEDEVIYEMDVRDFSIDPNSGMKNKGKYLALTEKGTKGPDNVKTGIDSLKQLGITHVQLMPVFASNSVDETDPTQDNWGYDPRNYDVPEGQYATNANGNARIKEFKEMVLSLHREHIGVNMDVVYNHTFATQISDFDKIVPEYYYRTDDAGNYTNGSGTGNEIAAERPMVQKFIIDSLKYWVNEYHIDGFRFDLMALLGKDTMSKAASELHAINPGIALYGEPWTGGTSALPDDQLLTKGAQKGMGVAVFNDNLRNALDGNVFDSSAQGFATGATGLTDAIKNGVEGSINDFTSSPGETINYVTSHDNYTLWDKIALSNPNDSEADRIKMDELAQAVVMTSQGVPFMQGGEEMLRTKGGNDNSYNAGDAVNEFDWSRKAQYPDVFNYYSGLIHLRLDHPAFRMTTANEINSHLQFLNSPENTVAYELTDHVNKDKWGNIIVVYNPNKTVATINLPSGKWAINATSGKVGESTLGQAEGSVQVPGISMMILHQEVSPDHGKK

SEQ ID NO: 4 - protein, 559 aa, Gloeophyllum trabeum
QSVDSYVGSEGPIAKAGVLANIGPNGSKASGAAAGVVVASPSKSDPDYWYTWTRDSSLVFKSLIDQYTTGIDSTSSLRSLIDSFVIAEANIQQVPNPSGTLTTGGLGEPKFNVDETAFTGPWGRPQRDGPALRATALITYGNWLLSNGNTTWVTSTLWPIIQNDLNYVVQYWNQTTFDLWEEVNSSSFFTTAVQHRALREGAAFATKIGQTSSVSSYTTQAANLLCFLQSYWNPTSGYITANTGGGRSGKDANTLLASIHTYDPSAGCDATTFQPCSDKALSNLKVYVDSFRSVYSINSGIASNAAVATGRYPEDSYQGGNPWYLTTFAVAEQLYDALNVWAAQGSLNVTSISLPFFQQFSSSVTAGTYASSSTTYTTLTSAIKSFADGFVAINAQYTPSNGGLAEQFSRSNGAPVSAVDLTWSYASALTAFEARNNTQFAGWGAVGLTVPTSCSSNSGGGGGSTVAVTFNVNAQTVWGENIYITGSVDALSNWSPDNALLLSSANYPTWSITVNLPASTAIQYKYIRKNNGAVTWESDPNNSITTPASGSVTENDTWR

SEQ ID NO: 5 - protein, 583 aa, Rhizomucor pusillus
ATSDDWKGKAIYQLLTDRFGRADDSTSNCSNLSNYCGGTYEGITKHLDYISGMGFDAIWISPIPKNSDGGYHGYWATDFYQLNSNFGDESQLKALIQAAHERDMYVMLDVVANHAGPTSNGYSGYTFDDASLYHPKCTIDYNNQTSIEQCWVADELPDIDTENSDNVAILNDIVSGWVGNYSFDGIRIDTVKHIRKDFWTGYAEAAGVFATGEVFNGDPAYVGPYQKYLPSLINYPMYYALNDVFVSKSKGFSRISEMLGSNRNAFEDTSVLTTFVDNHDNPRFLNSQSDKALFKNALTYVLLGEGIPIVYYGSEQGFSGGADPANREVLWTTNYDTSSDLYQFIKTVNSVRMKSNKAVYMDIYVGDNAYAFKHGDALVVLNNYGSGSTNQVSFSVSGKFDSGASLMDIVSNITTTVSSDGTVTFNLKDGLPAIFTSATGGTTTTATPTGSGSVTSTSKTTATASKTSTSTSSTSCTTPTAVAVTFDLTATTTYGENIYLVGSISQLGDWETSDGIALSADKYTSSDPLWYVTVTLPAGESFEYKFIRIESDDSVEWESDPNREYTVPQACGTSTATVTDTWR

SEQ ID NO: 6 - protein, 573 aa, Gloeophyllum sepiarium
MYRFLVCALGLAASVLAQSVDSYVSSEGPIAKAGVLANIGPNGSKASGASAGVVVASPSTSDPDYWYTWTRDSSLVFKSLIDQYTTGIDSTSSLRTLIDDFVTAEANLQQVSNPSGTLTTGGLGEPKFNVDETAFTGAWGRPQRDGPALRSTALITYGNWLLSNGNTSYVTSNLWPIIQNDLGYVVSYWNQSTYDLWEEVDSSSFFTTAVQHRALREGAAFATAIGQTSQVSSYTTQADNLLCFLQSYWNPSGGYITANTGGGRSGKDANTLLASIHTYDPSAGCDAATFQPCSDKALSNLKVYVDSFRSVYSINSGVASNAAVATGRYPEDSYQGGNPWYLTTFAVAEQLYDALNVWESQGSLEVTSTSLAFFQQFSSGVTAGTYSSSSSTYSTLTSAIKNFADGFVAINAKYTPSNGGLAEQYSKSDGSPLSAVDLTWSYASALTAFEARNNTQFAGWGAAGLTVPSSCSGNSGGPTVAVTFNVNAETVWGENIYLTGSVDALENWSADNALLLSSANYPTWSITVNLPASTAIEYKYIRKNNGAVTWESDPNNSITTPASGSTTENDTWR

SEQ ID NO: 7 - protein, 573 aa, Gloeophyllym sepiarium
MYRFLVCALGLAASVLAQSVDSYVSSEGPIAKAGVLANIGPNGSKASGASAGVVVASPSTSDPDYWYTWTRDSSLVFKSLIDQYTTGIDSTSSLRTLIDDFVTAEANLQQVSNPSGTLTTGGLGEPKFNVDETAFTGAWGRPQRDGSALRSTALITYGNWLLSNGNTSYVTSKLWPIIQNDLGYVVSYWNQSTYDLWEEVDSSSFFTTAVQHRALREGAAFATAIGQTSQVSSYTTQADNLLCFLQSYWNPSGGYITANTGGGRSGKDANTLLASIHTYDPSAGCDAATFQPCSDKALSNLKVYVDSFRSVYSINSGIASNAAVATGRYPEDSYQGGNPWYLTTFAVAEQLYDALNVWESQGSLEVTSTSLAFFQQFSSGVTAGTYSSSSSTYSTLTSAIKSFADGFVTINAKYTPSNGGLAEQYSKSDGSPLSAVDLTWSYASALTAFEARNDTQFAGWGAAGLTVPSSCSGNSGGPTVAVTFNVNAETVWGENIYLTGSVDALENWSADNALLLSSANYPTWSITVNLPASTAIEYKYIRKNNGAVTWESDPNNSITTPASGSTTENDTWR

SEQ ID NO: 8 - protein, 573 aa, Gloeophyllum trabeum
MYRFLVCALGLAATVLAQSVDSYVSSEGPIAKAGVLANIGPNGSKASGASAGVVVASPSTSDPDYWYTWTRDSSLVFKSLIDQYTTGIDSTSSLRTLIDDFVTAEANLQQVSNPSGTLTTGGLGEPKFNVDETAFTGAWGRPQRDGPALRSTALITYGNWLLSNGNTSYVTSILWPIIQNDLGYVVSYWNQSTYDLWEEVDSSSFFTTAVQHRALREGAAFATAIGQTSQVSSYTTQADNLLCFLQSYWNPSGGYITANTGGGRSGKDANTLLASIHTYDPSAGCDAATFQPCSDKALSNLKVYFDSFRSVYSINSGVASNAAVATGRYPEDSYQGGNPWYLTTFAVAEQLYDALNVWESQGSLEVTSTSLAFFQQFSSGVTAGTYSSSSSTYSTLTSAIKNFADGFVAINAKYTPSNGGLAEQYSKSDGSPLSAVDLTWSYASALTAFEARNNTQFAGWGAAGLTVPSSCSGNSGGPTVAVTFNVNAETVWGENIYLTGSVDALENWSADNALLLSSANYPTWSITVNLPASTAIEYKYIRKNNGAVTWESDPNNSITTPASGSTTENDTWR

SEQ ID NO: 9 - protein, 573 aa, Gloeophyllum sepiarium
MYRFLVCALGLAASVLAQSVDSYVSSEGPIAKAGVLANIGPNGSKASGASAGVVVASPSTSDPDYWYTWTRDSSLVFKSLIDQYTTGIDSTSSLRTLIDDFVTAEANLQQVSNPSGTLTTGGLGEPKFNVDETAFTGAWGRPQRDGPALRSTALITYGNWLLSNGNTSYVTSNLWPIIQNDLGYVVSYWNQSTYDLWEEVDSSSFFTTAVQHRALREGAAFATAIGQTSQVSSYTTQADNLLCFLQSYWNPSGGYITANTGGGRSGKDANTLLASIHTYDPSAGCDAATFQPCSDKALSNLKVYVDSFRSVYSINSGIASNAAVATGRYPEDSYQGGNPWYLTTFAVAEQLYDALNVWELQGSLEVTSTSLAFFQQFSSGVTAGTYSSSSSTYSTLTSAIKSFADGFVAINAKYTPSNGGLAEQYSKSDGSPLSAVDLTWSYASALTAFEARNDTQFAGWGAASLTVPSSCSGNSGGPTVAVTFNVNAETVWGENIYLTGSVDALENWSADNALLLSSANYPTWSITVNLPASTAIEYKYIRKNNGAVTWESDPNNSITTPASGSTTENDTWR

SEQ ID NO: 10 - protein, 573 aa, Gloeophyllum sepiarium
MYRFLVCALGLAATVLAQSVDSYVSSEGPVAKAGVLANIGPNGSKASGASAGVVVASPSTSDPDYWYTWTRDSSLVFKSLIDQYTTGIDSTSSLRTLIDDFVTAEANLQQVSNPSGTLTTGGLGEPKFNVDETAFTGAWGRPQRDGPALRSTALITYGNWLLSNGNTSYVTSNLWPIIQNDLGYVVSYWNQSTYDLWEEVDSSSFFTTAVQHRALREGAAFATAIGQTSQVSSYTTQADNLLCFLQSYWNPSGGYITANTGGGRSGKDANTLLASIHTYDPSAGCDAATFQPCSDKALSNLKVYVDSFRSIYSINSGIASNAAVATGRYPEDSYQGGNPWYLTTFAVAEQLYDALNVWESQGSLEVTSTSLAFFQQFSSGVTAGTYSSSSSTYSTLTSAIKSFADGFVAINAKYTPSNGGLAEQYSKSDGSPLSAVDLTWSYASALTAFEARNDTQFAGWGAAGLTVPSSCSGNSGGPTVAVTFNVNAETVWGENIYLTGSVDALENWSADNALLLSSANYPTWSITVNLPASTAIEYKYIRKNNGAVTWESDPNNSITTPASGSTTENDTWR

SEQ ID NO: 11 - protein, 573 aa, Gloeophyllum sp
MYRFLVCALGLAATVLAQSVDSYVSSEGPVAKAGVLANIGPNGSKASGASAGVVVASPSTSDPDYWYTWTRDSSLVFKSLIDQYTTGIDSTSSLRTLIDDFVTAEANLQQVSNPSGTLTTGGLGEPKFNVDETAFTGAWGRPQRDGPALRSTALITYGNWLLSNGNTSYVTSNLWPIIQNDLGYVVSYWNQSTYDLWEEVDSSSFFTTAVQHRALREGAAFATAIGQTSQVSSYTTQADNLLCFLQSYWNPSGGYITANTGGGRSGKDANTLLASIHTYDPSAGCDAATFQPCSDKALSNLKVYVDSFRSIYSINSGIASNAAVATGRYPEDSYQGGNPWYLTTFAVAEQLYDALNVWESQGSLEVTSTSLAFFQQFSSGVTAGTYSSSSSTYSTLTSAIKSFADGFVAINAKYTPSNGGLAEQYSKSDGSPLSAVDLTWSYASALTAFEARNDTQFAGWGAAGLTVPSSCSGNSGGPTVAVTFNVNAETVWGENIYLTGSVDALENWSADNALLLSSVNYPTWSITVNLPASTAIEYKYIRKNNGAVTWESDPNNSITTPASGSTTENDTWR

SEQ ID NO: 12 - protein, 573 aa, Gloeophyllum trabeum
MYRFLVCALGLAASVLAQSVDSYVSSEGPIAKAGVLANIGPNGSKASGASAGVVVASPSTSDPDYWYTWTRDSSLVFKSLIDQYTTGIDGTSSLRTLIDDFVTAEANLQQVSNPSGTLTTGGLGEPKFNVDETAFTGAWGRPQRDGPALRSTALITYGNWLLSNGNTSYVTSNLWPIIQNDLGYVVSYWNQSTYDLWEEVDSSSFFTTAVQHRALREGAAFATAIGQTSQVSSYTTQADNLLCFLQSYWNPSGGYITANTGGGRSGKDANTLLASIHTYDPSAGCDAATFQPCSDKALSNLKVYVDSFRSVYSINSGIASNAAVATGRYPEDSYQGGNPWYLTTFAVAEQLYDALNVWESQGSLEVTSTSLAFFQQFSSGVTAGTYSSSSSTYSTLTSAIKSFADGFVAVNAKYTPSNGGLAEQYSKSDGSPLSAVDLTWSYASALTAFEARNNTQFAGWGAAGLTVPSSCSGNSGGPTVAVTFNVNAETVWGENIYLTGSVDALENWSADNALLLSSANYPTWSITVNLPASTAIEYKYIRKNNGAVTWESDPNNSITTPASGSTTENDTWR

SEQ ID NO: 13 - protein, 576 aa, Gloeophyllum trabeum
MYRFLVCALGLLGTVLAQSVDSYVGSEGPIAKAGVLANIGPNGSKASGAAAGVVVASPSKSDPDYWYTWTRDSSLVFKSLIDQYTTGIDSTSSLRSLIDSFVIAEANIQQVSNPSGTLTTGGLGEPKFNVDETAFTGAWGRPQRDGPALRATALITYGNWLLSNGNTTWVTSTLWPIIQNDLNYVVQYWNQTTFDLWEEVNSSSFFTTAVQHRALREGAAFATKIGQTSSVSSYTTQAANLLCFLQSYWNPTSGYITANTGGGRSGKDANTLLASIHTYDPSAGCDATTFQPCSDKALSNLKVYVDSFRSVYSINSGIASNAAVATGRYPEDSYQGGNPWYLTTFAVAEQLYDALNVWAAQGSLNVTSISLPFFQQFSSSVTAGTYASSSTTYTTLTSAIKSFADGFVAINAQYTPSNGGLAEQFSRSNGSPVSAVDLTWSYASALTAFEARNNTQFAGWGAVGLTVPTSCSSNSGGGGGSTVAVTFNVNAQTVWGENIYITGSVDALSNWSPDNALLLSSANYPTWSITVNLPASTAIQYKYIRKNNGAVTWESDPNNSITTPASGSVTENDTWR

SEQ ID NO: 14 - protein, 576 aa, Gloeophyllum trabeum
MYRFLVCALGLLGTVLAQSVDSYVGSEGPIAKAGVLANIGPNGSKASGAAAGVVVASPSKSDPDYWYTWTRDSSLVFKSLIDQYTTGIDSTSSLRSLIDSFVIAEANIQQVSNPSGTLTTGGLGEPKFNVDETAFTGAWGRPQRDGPALRATALITYGNWLLSNGNTTWVTSTLWPIIQNDLNYVVQYWNQTTFDLWEEVNSSSFFTTAVQHRALREGAAFATKIGQTSSVSSYTTQAANLLCFLQSYWNPTSGYITANTGGGRSGKDANTLLASIHTYDPSAGCDATTFQPCSDKALSNLKVYVDSFRSVYSINSGIASNAAVATGRYPEDSYQGGNPWYLTTFAVAEQLYDALNVWAAQGSLNVTSISLPFFQQFSSSVTAGTYASSSTTYTTLTSAIKSFADGFVAINAQYTPSNGGLAEQFSRSNGAPVSAVDLTWSYASALTAFEARNNTQFAGWGAVGLTVPTSCSSNSGGGGGSTVAVTFNVNAQTVWGENIYITGSVDALSNWSPDNALLLSSANYPTWSITVNLPASTAIQYKYIRKNNGAVTWESDPNNSITTPASGSVTENDTWR

SEQ ID NO: 15 - protein, 618 aa, Talaromyces emersonii
MASLVAGALCILGLTPAAFARAPVAARATGSLDSFLATETPIALQGVLNNIGPNGADVAGASAGIVVASPSRSDPNYFYSWTRDAALTAKYLVDAFIAGNKDLEQTIQQYISAQAKVQTISNPSGDLSTGGLGEPKFNVNETAFTGPWGRPQRDGPALRATALIAYANYLIDNGEASTADEIIWPIVQNDLSYITQYWNSSTFDLWEEVEGSSFFTTAVQHRALVEGNALATRLNHTCSNCVSQAPQVLCFLQSYWTGSYVLANFGGSGRSGKDVNSILGSIHTFDPAGGCDDSTFQPCSARALANHKVVTDSFRSIYAINSGIAEGSAVAVGRYPEDVYQGGNPWYLATAAAAEQLYDAIYQWKKIGSISITDVSLPFFQDIYPSAAVGTYNSGSTTFNDIISAVQTYGDGYLSIVEKYTPSDGSLTEQFSRTDGTPLSASALTWSYASLLTASARRQSVVPASWGESSASSVPAVCSATSATGPYSTATNTVWPSSGSGSSTTTSSAPCTTPTSVAVTFDEIVSTSYGETIYLAGSIPELGNWSTASAIPLRADAYTNSNPLWYVTVNLPPGTSFEYKFFKNQTDGTIVWEDDPNRSYTVPAYCGQTTAILDDSWQ

SEQ ID NO: 16 - protein, 828 aa, Artificial sequence
  Hybrid pullulanase
DSTSTEVIVHYHRFDSNYANWDLWMWPYQPVNGNGAAYEFSGKDDFGVKADVQVPGDDTQVGLIVRTNDWSQKNTSDDLHIDLTKGHEIWIVQGDPNIYYNLSDAQAAATPKVSNAYLDNEKTVLAKLTNPMTLSDGSSGFTVTDKTTGEQIPVTAATNANSASSSEQTDLVQLTLASAPDVSHTIQVGAAGYEAVNLIPRNVLDSSQYYYSGDDLGNTYTHKATTFKVWAPTSTQVNVLLYNSATGSVTKTVPMTASGHGVWEATVNQNLENWYYMYEVTGQGSTRTAVDPYATAIAPNGTRGMIVDLAKTDPAGWNSDKHITPKNIEDEVIYEMDVRDFSIDPNSGMKNKGKYLALTEKGTKGPDGVKTGIDSLKQLGITHVQLMPVFAFASVDETDPTQDNWGYDPRNYDVPEGQYATNANGTARIKEFKEMVLSLHREHIGVNMDVVYNHTFATQISDFDKIVPEYYYRTDDAGNYTNGSGTGNEIASERPMVQKFIIDSLKYWVNEYHIDGFRFDLMALLGKDTMSKAASELHAINPGIALYGEPWTGGTSALPEDQLLTKGAQKGMGVAVFNDNLRNALDGNVFDSSAQGFATGATGLTDAIKNGVEGSINDFTSSPGETINYVTSHDNYTLWDKIALSNPNDSEADRIKMDELAQAVVMTSQGVPFMQGGEEMLRTKGGNDNSYNAGDTVNEFDWSRKAQYPDVFNYYSGLIHLRLDHPAFRMTTANEINSHLQFLNSPENTVAYELTDHVNKDKWGNIIVVYNPNKTAATINLPSGKWAINATSGKVGESTLGQAEGSVQVPGISMMILHQEVSPDHGKK

SEQ ID NO: 17 - protein, 928 aa, Artificial sequence
  hybrid pullulanase
ASSTEVIVHYHRFDANYANWDLWMWPYQPVNGNGAAYEFSGTDEFGVTADVQVPGDNTQVGLIVRKNDWSQKNTPDDLHIDLSKGHEVWINQGDPTIYYNLNDAEAAAVPAVSNAYLDNEKTVLAKLSSPMTLTDGASGFTVTDETTGEQIPVVSAESANPVTAVLVGDFQQALGASGNWSPDDDHTKLSKINSNLYQFTGTLPAGTYQYKVALDHSWSASYPNNNVNLTVPAGGTKVTFTYIPSTHQVFDSINNPDQTFPSSSAGTQSDLVQLTLASAPDITHDLQVVADGYKGGKILPRNVLNLPRYYYSGNDLGNVYSNKATAFRVWAPTASDVQLLLYNSETGPVTKQLEMQKSDNGTWKLKVPGNLKNWYYLYQVTVNGKTQTAVDPYVRAISVNATRGMIVDLEDTNPPGWKEDHQQTPANPVDEVIYEVHVRDFSIDANSGMKNKGKYLAFTEHGTKGPDGVKTGIDSLKELGINAVQLQPIEEFASIDETQPNMYNWGYDPRNYNVPEGAYATTPEGTARITEFKQLIQSIHKDRIAINMDVVYNHTFSTLISDFDKIVPQYYYRTDDAGNYTNGSGVGNEFATEHPMARKFVLDSLKYWVTQYHIDGFRFDLMALLGKNTMAEASKELHAINPGIVLYGEPWTGGTSGITGDQLLTKGVQKGLGIGVFNDNLRNALDGNVFDSSAQGFATGATGLTDAIKRGVEGSINDFTSSPSETINYVSCHDNYTLWDKIALSNPNDSEADRIKMDELAQAVVMTSQGVPFMQGGEEMLRTKGGNDNSYNAGDTVNEFDWSRKAQYPDVFNYYSGLIHLRLDHPAFRMTTANEINSHLQFLNSPENTVAYELTDHVNKDKWGNIIVVYNPNKTAATINLPSGKWAINATSGKVGESTLGQAEGSVQVPGISMMILHQEVSPDHGKK

SEQ ID NO: 18 - protein, 928 aa, Artificial sequence
  Hybrid pullulanase
ASSTEVIVHYHRFDANYANWDLWMWPYQPVNGNGAAYEFSGTDEFGVTADVQVPGDNTQVGLIVRKNDWSQKNTPDDLHIDLSKGHEVWINQGDPTIYYNLNDAEAAAVPAVSNAYLDNEKTVLAKLSSPMTLTDGASGFTVTDETTGEQIPVVSAESANPVTAVLVGDFQQALGASGNWSPDDDHTKLSKINSNLYQFTGTLPAGTYQYKVALDHSWSASYPNNNVNLTVPAGGTKVTFTYIPSTHQVFDSINNPDQTFPSSSAGTQSDLVQLTLASAPDITHDLQVVADGYKGGKILPRNVLNLPRYYYSGNDLGNVYSNKATAFRVWAPTASDVQLLLYNSETGPVTKQLEMQKSDNGTWKLKVPGNLKNWYYLYQVTVNGKTQTAVDPYVRAISVNATRGMIVDLEDTNPPGWKEDHQQTPANPVDEVIYEVHVRDFSIDANSGMKNKGKYLAFTEHGTKGPDGVKTGIDSLKELGINAVQLQPIEEFASIDETQPNMYNWGYDPRNYNVPEGAYATTPEGTARITEFKQLIQSIHKDRIAINMDVVYNHTFATQISDFDKIVPEYYYRTDDAGNYTNGSGTGNEIAAERPMVQKFIIDSLKYWVNEYHIDGFRFDLMALLGKDTMSKAASELHAINPGIALYGEPWTGGTSALPEDQLLTKGAQKGMGVAVFNDNLRNALDGNVFDSSAQGFATGATGLTDAIKRGVEGSINDFTSSPSETINYVSCHDNYTLWDKIALSNPNDSEADRIKMDELAQAVVMTSQGVPFMQGGEEMLRTKGGNDNSYNAGDTVNEFDWSRKAQYPDVFNYYSGLIHLRLDHPAFRMTTANEINSHLQFLNSPENTVAYELTDHVNKDKWGNIIVVYNPNKTAATINLPSGKWAINATSGKVGESTLGQAEGSVQVPGISMMILHQEVSPDHGKK

SEQ ID NO: 19 - protein, 471 aa, Rhizomucor pusillus
MKFSISLSAAIVLFAAATSLASPLPQQQRYGKRATSDDWKSKAIYQLLTDRFGRADDSTSNCSNLSNYCGGTYEGITKHLDYISGMGFDAIWISPIPKNSDGGYHGYWATDFYQLNSNFGDESQLKALIQAAHERDMYVMLDVVANHAGPTSNGYSGYTFGDASLYHPKCTIDYNDQTSIEQCWVADELPDIDTENSDNVAILNDIVSGWVGNYSFDGIRIDTVKHIRKDFWTGYAEAAGVFATGEVFNGDPAYVGPYQKYLPSLINYPMYYALNDVFVSKSKGFSRISEMLGSNRNAFEDTSVLTTFVDNHDNPRFLNSQSDKALFKNALTYVLLGEGIPIVYYGSEQGFSGGADPANREVLWTTNYDTSSDLYQFIKTVNSVRMKSNKAVYMDIYVGDNAYAFKHGDALVVLNNYGSGSTNQVSFSVSGKFDSGASLMDIVSNITTTVSSDGTVTFNLKDGLPAIFTSA

SEQ ID NO: 20 - protein, 514 aa, B. stearothermophilus
AAPFNGTMMQYFEWYLPDDGTLWTKVANEANNLSSLGITALWLPPAYKGTSRSDVGYGVYDLYDLGEFNQKGAVRTKYGTKAQYLQAIQAAHAAGMQVYADVVFDHKGGADGTEWVDAVEVNPSDRNQEISGTYQIQAWTKFDFPGRGNTYSSFKWRWYHFDGVDWDESRKLSRIYKFRGIGKAWDWEVDTENGNYDYLMYADLDMDHPEVVTELKSWGKWYVNTTNIDGFRLDAVKHIKFSFFPDWLSDVRSQTGKPLFTVGEYWSYDINKLHNYIMKTNGTMSLFDAPLHNKFYTASKSGGTFDMRTLMTNTLMKDQPTLAVTFVDNHDTEPGQALQSWVDPWFKPLAYAFILTRQEGYPCVFYGDYYGIPQYNIPSLKSKIDPLLIARRDYAYGTQHDYLDHSDIIGWTREGVTEKPGSGLAALITDGPGGSKWMYVGKQHAGKVFYDLTGNRSDTVTINSDGWGEFKVNGGSVSVWVPRKTTVSTIAWSITTRPWTDEFVRWTEPRLVAW

SEQ ID NO: 21 - protein, 483 aa, Bacillus licheniformis [sequence omitted]

SEQ ID NO: 22 - protein, 483 aa, Bacillus amyloliquefaciens
VNGTLMQYFEWYTPNDGQHWKRLQNDAEHLSDIGITAVWIPPAYKGLSQSDNGYGPYDLYDLGEFQQKGTVRTKYGTKSELQDAIGSLHSRNVQVYGDVVLNHKAGADATEDVTAVEVNPANRNQETSEEYQIKAWTDFRFPGRGNTYSDFKWHWYHFDGADWDESRKISRIFKFRGEGKAWDWEVSSENGNYDYLMYADVDYDHPDVVAETKKWGIWYANELSLDGFRIDAAKHIKFSFLRDWVQAVRQATGKEMFTVAEYWQNNAGKLENYLNKTSFNQSVFDVPLHFNLQAASSQGGGYDMRRLLDGTVVSRHPEKAVTFVENHDTQPGQSLESTVQTWFKPLAYAFILTRESGYPQVFYGDMYGTKGTSPKEIPSLKDNIEPILKARKEYAYGPQHDYIDHPDVIGWTREGDSSAAKSGLAALITDGPGGSKRMYAGLKNAGETWYDITGNRSDTVKIGSDGWGEFHVNDGSVSIYVQK

SEQ ID NO: 23 - protein, 483 aa, Artificial sequence
  Recombinant alpha-amylase conjugate
AAVNGTLMQYFEWYTPNDGQHWKRLQNDAEHLSDIGITAVWIPPAYKGTSQADVGYGAYDLYDLGEFHQKGTVRTKYGTKGELQSAIKSLHSRDINVYGDVVINHKGGADATEDVTAVEVDPADRNRVISGEHLIKAWTHFHFPGRGSTYSDFKWHWYHFDGTDWDESRKLNRIYKFQGKAWDWEVSNENGNYDYLMYADIDYDHPDVAAEIKRWGTWYANELQLDGFRLDAVKHIKFSFLRDWVNHVREKTGKEMFTVAEYWQNDLGALENYLNKTNFNHSVFDVPLHYQFHAASTQGGGYDMRKLLNGTVVSKHPLKSVTFVDNHDTQPGQSLESTVQTWFKPLAYAFILTRESGYPQVFYGDMYGTKGDSQREIPALKHKIEPILKARKQYAYGAQHDYFDHHDIVGWTREGDSSVANSGLAALITDGPGGAKRMYVGRQNAGETWHDITGNRSEPVVINSEGWGEFHVNGGSVSIYVQR

SEQ ID NO: 24 - protein, 483 aa, Artificial sequence
  Bacillus hybrid alpha-amylase
AAVNGTLMQYFEWYTPNDGQHWKRLQNDAEHLSDIGITAVWIPPAYKAISQADVGYGAYDLYDLGEFHQKGTVRTKYGTKGELQSAIKSLHSRDINVYGDVVINHKAGADATEDVTAVEVDPADRNRVISGEHLIKAWTHFHFPGRGSTYSDFKWYWYHFDGTDWDESRKLNRIYKFQGKTWDWEVSNEFGNYDYLMYADFDYDHPDVVAEIKRWGTWYANELQLDGFRLDAVKHIKFSFLRDWVNHVREKTGKEMFTVAEYWSNDLGALENYLNKTNFNHSVFDVPLHYQFHAASTQGGGYDMRKLLNGTVVSKHPLKSVTFVDNHDTQPGQSLESTVQTWFKPLAYAFILTRESGYPQVFYGDMYGTKGDSQREIPALKHKIEPILKARKQYAYGAQHDYFDHHDIVGWTREGDSSVANSGLAALITDGPGGAKRMYVGRQNAGETWHDITGNRSEPVVINSEGWGEFHVNGGSVSIYVQR

SEQ ID NO: 25 - protein, 483 aa, Artificial sequence
  Bacillus hybrid alpha-amylase variant
AAVNGTLMQYFEWYTPNDGQHWKRLQNDAEHLSDIGITAVWIPPAYKAISQADVGYGAYDLYDLGEFWQKGTVRTKYGTKGELQSAIKSLHSRDINVYGDVVINHKAGADATEDVTAVEVDPADRNRVISGEHLIKAWTHFHFPGRGSTYSDFKWYWYHFDGTDWDESRKLNRIYLFQGKTWDWPVSNEFGNYDYLMYADYDYDYPDVVAEITRWGTWYANELQLDGFRLDAVKHIKFSFLRDWVNHVREKTGKEMFTVAEYWSNDLGALENYLNKTNFNHSVFDVPLHYQFHAASTQGGGYDMRKLLNGTVVSKHPLKSVTFVDNHDTQPGQSLESTVQTWFKPLAYAFILTRESGYPSVFYGDMYGTKGDSQREIPALKHKIEPILKARKQYAYGAQHDYFDHHDIVGWTREGVSSVANSGLAALITDGPGGAKWMYVGRQNAGETWHDITGNRSEPVVINSEGWGEFHVNGGSVSIYVQR